European Patent Specification EP 3 712 609 B1, published December 27, 2023. Title: ANALYSIS METHOD FOR GLYCAN HAVING ACID GROUP. Applicant: JCR Pharmaceuticals Co., Ltd. The sequence listing filed with the application follows.

SEQUENCE LISTING (8 sequences)

SEQ ID NO: 1 - protein, 219 aa, Artificial Sequence
  amino acid sequence of the light-chain of humanized anti-hTfR antibody
DIVMTQTPLSLSVTPGQPASISCRSSQSLVHSNGNTYLHWYLQKPGQSPQLLIYKVSNRFSGVPDRFSGSGSGTDFTLKISRVEAEDVGVYYCSQSTHVPWTFGQGTKVEIKRTVAAPSVFIFPPSDEQLKSGTASVVCLLNNFYPREAKVQWKVDNALQSGNSQESVTEQDSKDSTYSLSSTLTLSKADYEKHKVYACEVTHQGLSSPVTKSFNRGEC

SEQ ID NO: 2 - protein, 448 aa, Artificial Sequence
  amino acid sequence of the heavy-chain of humanized anti-hTfR antibody
EVQLVQSGAEVKKPGESLKISCKGSGYSFTNYWLGWVRQMPGKGLEWMGDIYPGGDYPTYSEKFKVQVTISADKSISTAYLQWSSLKASDTAMYYCARSGNYDEVAYWGQGTLVTVSSASTKGPSVFPLAPSSKSTSGGTAALGCLVKDYFPEPVTVSWNSGALTSGVHTFPAVLQSSGLYSLSSVVTVPSSSLGTQTYICNVNHKPSNTKVDKKVEPKSCDKTHTCPPCPAPELLGGPSVFLFPPKPKDTLMISRTPEVTCVVVDVSHEDPEVKFNWYVDGVEVHNAKTKPREEQYNSTYRVVSVLTVLHQDWLNGKEYKCKVSNKALPAPIEKTISKAKGQPREPQVYTLPPSRDELTKNQVSLTCLVKGFYPSDIAVEWESNGQPENNYKTTPPVLDSDGSFFLYSKLTVDKSRWQQGNVFSCSVMHEALHNHYTQKSLSLSPGK

SEQ ID NO: 3 - DNA, 20 bp, Artificial Sequence
  Primer Hyg-Sfi5', synthetic sequence
gaggccgcctcggcctctga

SEQ ID NO: 4 - DNA, 29 bp, Artificial Sequence
  Primer Hyg-BstX3', synthetic sequence
aaccatcgtgatgggtgctattcctttgc

SEQ ID NO: 5 - DNA, 740 bp, Artificial Sequence
  nucleotide seuquence encoding amino acid sequence of the light-chain of humanized anti-hTfR antibody, synthetic sequence
acgcgtgccgccaccatgggctggagctggattctgctgttcctcctgagcgtgacagcaggagtgcacagcgacatcgtgatgacccagactcccctgagcctgagcgtgacacctggccagcctgccagcatcagctgcagaagctctcagagcctggtgcacagcaacggcaacacctacctgcactggtatctgcagaagcccggccagagccctcagctgctgatctacaaggtgtccaacagattcagcggcgtgcccgacagattctccggcagcggctctggcaccgacttcaccctgaagatttccagagtggaagccgaggacgtgggcgtgtactactgcagccagagcacccacgtgccctggacattcggccagggcaccaaggtggaaatcaagagaaccgtggccgctcccagcgtgttcatcttcccacctagcgacgagcagctgaagtccggcacagcctctgtcgtgtgcctgctgaacaacttctacccccgcgaggccaaggtgcagtggaaggtggacaacgccctgcagagcggcaacagccaggaaagcgtgaccgagcaggactccaaggacagcacctacagcctgagcagcaccctgaccctgagcaaggccgactacgagaagcacaaggtgtacgcctgcgaagtgacccaccagggcctgtctagccccgtgaccaagagcttcaacagaggcgagtgctaagcggccgc

SEQ ID NO: 6 - protein, 525 aa, Homo sapiens
SETQANSTTDALNVLLIIVDDLRPSLGCYGDKLVRSPNIDQLASHSLLFQNAFAQQAVCAPSRVSFLTGRRPDTTRLYDFNSYWRVHAGNFSTIPQYFKENGYVTMSVGKVFHPGISSNHTDDSPYSWSFPPYHPSSEKYENTKTCRGPDGELHANLLCPVDVLDVPEGTLPDKQSTEQAIQLLEKMKTSASPFFLAVGYHKPHIPFRYPKEFQKLYPLENITLAPDPEVPDGLPPVAYNPWMDIRQREDVQALNISVPYGPIPVDFQRKIRQSYFASVSYLDTQVGRLLSALDDLQLANSTIIAFTSDHGWALGEHGEWAKYSNFDVATHVPLIFYVPGRTASLPEAGEKLFPYLDPFDSASQLMEPGRQSMDLVELVSLFPTLAGLAGLQVPPRCPVPSFHVELCREGKNLLKHFRFRDLEEDPYLPGNPRELIAYSQYPRPSDIPQWNSDKPSLKDIKIMGYSIRTIDYRYTVWVGFNPDEFLANFSDIHAGELYFVDSDPLQDHNMYNDSQGGDLFQLLMP

SEQ ID NO: 7 - DNA, 3008 bp, Artificial Sequence
  nucleotide seuquence encoding amino acid sequence of fused protein of the heavy-chain of humanized anti-hTfR antibody and hI2S, synthetic sequence
acgcgtgccgccaccatgggctggagctggattctgctgttcctcctgagcgtgacagcaggagtgcacagcgaggtgcaactagtgcagtctggagcagaggtgaaaaagcccggggagtctctgaagatcagctgtaagggttctggatacagctttatgaactactggctgggatgggtgcgccagatgcccgggaaaggcctggagtggattggggacatctaccccggcggagactaccctacatacagcgagaagttcaaggtcaaggccatcatctcagccgacacgtccatcagcaccgtctacctgcagttgagcagcctgaaggcctcggacaccgccatgtatttctgtgcgagatcaggcaattacgacgaagtggcctactggggccaaggaaccctggtcaccgtctcctcagctagcaccaagggcccatcggtcttccccctggcaccctcctccaagagcacctctgggggcacagcggccctgggctgcctggtcaaggactacttccccgaaccggtgacggtgtcgtggaactcaggcgccctgaccagcggcgtgcacaccttcccggctgtcctacagtcctcaggactctactccctcagcagcgtggtgaccgtgccctccagcagcttgggcacccagacctacatctgcaacgtgaatcacaagcccagcaacaccaaggtggacaagaaagttgagcccaaatcttgtgacaaaactcacacgtgcccaccgtgcccagcacctgaactcctggggggtccgtcagtcttcctcttccccccaaaacccaaggacaccctcatgatctcccggacccctgaggtcacatgcgtggtggtggacgtgagccacgaagaccctgaggtcaagttcaactggtacgtggacggcgtggaggtgcataatgccaagacaaagccgcgggaggagcagtacaacagcacgtaccgggtggtcagcgtcctcaccgtcctgcaccaggactggctgaatggcaaggagtacaagtgcaaggtctccaacaaagccctcccagcccccatcgagaaaaccatctccaaagccaaagggcagccccgagaaccacaggtgtacaccctgcccccatcccgggatgagctgaccaagaaccaggtcagcctgacctgcctggtcaaaggcttctatcccagcgacatcgccgtggagtgggagagcaatgggcagccggagaacaactacaagaccacgcctcccgtgctggactccgacggctccttcttcctctacagcaagctcaccgtggacaagagcaggtggcagcaggggaacgtcttctcatgctccgtgatgcatgaggctctgcacaaccactacacgcagaagagcctctccctgtctccgggtaaaggatcttccgaaacgcaggccaactcgaccacagatgctctgaacgttcttctcatcatcgtggatgacctgcgcccctccctgggctgttatggggataagctggtgaggtccccaaatattgaccaactggcatcccacagcctcctcttccagaatgcctttgcgcagcaagcagtgtgcgccccgagccgcgtttctttcctcactggcaggagacctgacaccacccgcctgtacgacttcaactcctactggagggtgcacgctggaaacttctccaccatcccccagtacttcaaggagaatggctatgtgaccatgtcggtgggaaaagtctttcaccctgggatatcttctaaccataccgatgattctccgtatagctggtcttttccaccttatcatccttcctctgagaagtatgaaaacactaagacatgtcgagggccagatggagaactccatgccaacctgctttgccctgtggatgtgctggatgttcccgagggcaccttgcctgacaaacagagcactgagcaagccatacagttgttggaaaagatgaaaacgtcagccagtcctttcttcctggccgttgggtatcataagccacacatccccttcagataccccaaggaatttcagaagttgtatcccttggagaacatcaccctggcccccgatcccgaggtccctgatggcctaccccctgtggcctacaacccctggatggacatcaggcaacgggaagacgtccaagccttaaacatcagtgtgccgtatggtccaattcctgtggactttcagcggaaaatccgccagagctactttgcctctgtgtcatatttggatacacaggtcggccgcctcttgagtgctttggacgatcttcagctggccaacagcaccatcattgcatttacctcggatcatgggtgggctctaggtgaacatggagaatgggccaaatacagcaattttgatgttgctacccatgttcccctgatattctatgttcctggaaggacggcttcacttccggaggcaggcgagaagcttttcccttacctcgacccttttgattccgcctcacagttgatggagccaggcaggcaatccatggaccttgtggaacttgtgtctctttttcccacgctggctggacttgcaggactgcaggttccacctcgctgccccgttccttcatttcacgttgagctgtgcagagaaggcaagaaccttctgaagcattttcgattccgtgacttggaagaagatccgtacctccctggtaatccccgtgaactgattgcctatagccagtatccccggccttcagacatccctcagtggaattctgacaagccgagtttaaaagatataaagatcatgggctattccatacgcaccatagactataggtatactgtgtgggttggcttcaatcctgatgaatttctagctaacttttctgacatccatgcaggggaactgtattttgtggattctgacccattgcaggatcacaatatgtataatgattcccaaggtggagaccttttccagttgttgatgccttaagcggccgc

SEQ ID NO: 8 - protein, 975 aa, Artificial Sequence
  amino acid sequence of fused protein of the heavy-chain of humanized anti-hTfR antibody and hI2S
EVQLVQSGAEVKKPGESLKISCKGSGYSFMNYWLGWVRQMPGKGLEWIGDIYPGGDYPTYSEKFKVKAIISADTSISTVYLQLSSLKASDTAMYFCARSGNYDEVAYWGQGTLVTVSSASTKGPSVFPLAPSSKSTSGGTAALGCLVKDYFPEPVTVSWNSGALTSGVHTFPAVLQSSGLYSLSSVVTVPSSSLGTQTYICNVNHKPSNTKVDKKVEPKSCDKTHTCPPCPAPELLGGPSVFLFPPKPKDTLMISRTPEVTCVVVDVSHEDPEVKFNWYVDGVEVHNAKTKPREEQYNSTYRVVSVLTVLHQDWLNGKEYKCKVSNKALPAPIEKTISKAKGQPREPQVYTLPPSRDELTKNQVSLTCLVKGFYPSDIAVEWESNGQPENNYKTTPPVLDSDGSFFLYSKLTVDKSRWQQGNVFSCSVMHEALHNHYTQKSLSLSPGKGSSETQANSTTDALNVLLIIVDDLRPSLGCYGDKLVRSPNIDQLASHSLLFQNAFAQQAVCAPSRVSFLTGRRPDTTRLYDFNSYWRVHAGNFSTIPQYFKENGYVTMSVGKVFHPGISSNHTDDSPYSWSFPPYHPSSEKYENTKTCRGPDGELHANLLCPVDVLDVPEGTLPDKQSTEQAIQLLEKMKTSASPFFLAVGYHKPHIPFRYPKEFQKLYPLENITLAPDPEVPDGLPPVAYNPWMDIRQREDVQALNISVPYGPIPVDFQRKIRQSYFASVSYLDTQVGRLLSALDDLQLANSTIIAFTSDHGWALGEHGEWAKYSNFDVATHVPLIFYVPGRTASLPEAGEKLFPYLDPFDSASQLMEPGRQSMDLVELVSLFPTLAGLAGLQVPPRCPVPSFHVELCREGKNLLKHFRFRDLEEDPYLPGNPRELIAYSQYPRPSDIPQWNSDKPSLKDIKIMGYSIRTIDYRYTVWVGFNPDEFLANFSDIHAGELYFVDSDPLQDHNMYNDSQGGDLFQLLMP